European Patent Application EP 4 772 186 A1, published July 8, 2026. Title: USE AND COMPOSITION OF POSTBIOTIC OF LACTOBACILLUS PARACASEI ET-22. Applicant: Inner Mongolia Yili Industrial Group Co., Ltd. Application EP 24858371.8, filed August 19, 2024. The sequence listing filed with the application follows.

SEQUENCE LISTING (11 sequences)

SEQ ID NO: 1 - DNA, 19 bp, synthetic construct
  source 1..19: mol_type = other DNA
aagcgcgtctaggttatgt

SEQ ID NO: 2 - DNA, 23 bp, synthetic construct
  source 1..23: mol_type = other DNA
tgtagttccgcttacctctccag

SEQ ID NO: 3 - DNA, 22 bp, synthetic construct
  source 1..22: mol_type = other DNA
acgaactttgccgttattgtca

SEQ ID NO: 4 - DNA, 21 bp, synthetic construct
  source 1..21: mol_type = other DNA
agcaatgcagccaatctacaa

SEQ ID NO: 5 - DNA, 20 bp, synthetic construct
  source 1..20: mol_type = other DNA
cacaagctgacgctgctaga

SEQ ID NO: 6 - DNA, 21 bp, synthetic construct
  source 1..21: mol_type = other DNA
gttaccagctcttaaagcttg

SEQ ID NO: 7 - DNA, 21 bp, synthetic construct
  source 1..21: mol_type = other DNA
aatacaggaattgggcttgct

SEQ ID NO: 8 - DNA, 24 bp, synthetic construct
  source 1..24: mol_type = other DNA
cttcagttccataggctctcataa

SEQ ID NO: 9 - DNA, 20 bp, synthetic construct
  source 1..20: mol_type = other DNA
tcgtgcttatgagcgatgtc

SEQ ID NO: 10 - DNA, 20 bp, synthetic construct
  source 1..20: mol_type = other DNA
ggaagtcaccctcgtggata

SEQ ID NO: 11 - protein, 6 aa, synthetic construct
  MOD_RES 3: note = 4Hyp
GPPGAG